European Patent Application EP 4 527 465 A2, published March 26, 2025. Title: ANTI-GLYPICAN 3 ANTIBODIES. Applicant: Concept to Medicine Biotech Co., Ltd. Application WO. The sequence listing filed with the application follows.

SEQUENCE LISTING (76 sequences)

SEQ ID NO: 1 - protein, 115 aa, synthetic construct
QVQLQQSGAELVRPGASVTLSCKASGYTFSDYEMHWVKQTPVHGLEWIGAIDPETGGTAYNQKFKGKATLTADKSSSTAYMELRSLTSEDSAVYYCTRYYSYAYWGQGTLVTVSA

SEQ ID NO: 2 - protein, 112 aa, synthetic construct
DVVMTQSPLSLPVSLGDQASISCRSRQSLVHSNGNTYLQWYLQKPGQSPKLLIYKVSNRFSGVPDRFSGSGSGTDFTLKISRVEAEDLGVYFCFQSIHVPYTFGGGTKLEKK

SEQ ID NO: 3 - protein, 115 aa, synthetic construct
QVQLQQSGAELVRPGASVKLSCKALGYTFTDYEMHWVKQTPVHGLEWIGAIHPGSGGTAYNQKFKGKATLTADKFSSTGYMELSSLTSEDSAVYYCTRFYSYAYWGQGTLVTVSA

SEQ ID NO: 4 - protein, 112 aa, synthetic construct
DVVMTQTPLSLPVSLGDQASISCRSSQSLVHSNGNTYLQWYLQKPGQSPKLLIYKVSNRFSGVPDRFSGSGSGTDFILKISRVEAEDLGVYFCSQSIHVPYTFGGGTKLEIK

SEQ ID NO: 5 - protein, 115 aa, synthetic construct
QVQLQQSGAELVRPGASVTLSCKASGYTFTDYEMHWVKQTPVHGLEWIGAIGPETGSTAYNQRFKGKAIVTADKSSSTAYMELRSLTSEDSAVYYCTRYYSFAYWGQGTLVTVSA

SEQ ID NO: 6 - protein, 112 aa, synthetic construct
DVVMTQTPLSLPVSLGGQASISCRSSQSLVHSNGNTYLQWYLQKPGQSPKLLIFKVSNRFSGVPDRFSGSGSGTDFTLKISRVEAEDLGVYFCFQSIHVPYTFGGGTKLEIK

SEQ ID NO: 7 - protein, 115 aa, synthetic construct
QVQLQQSGAELVRPGASVTLSCKASGYTFTDYEIHWVKQTPVHGLEWIGAIDPATGDTAYTQKFKGKAILTADTSSNTVYMELRGLTSEDSAVHFCTRFYSYAYWGQGTLVTVSA

SEQ ID NO: 8 - protein, 112 aa, synthetic construct
DVVMTQTPLSLPVSLGDQASISCRSSQSLVHTNGHTYLQWYLQKSGQSPRLLIFKVSNRFSGVPDRFSGSGSGTDFKLKISRVEAEDLGVYFCSQSTHVPYTFGGGTKLEIK

SEQ ID NO: 9 - protein, 115 aa, synthetic construct
QVQLQQSGAELVRPGASVTLSCKASGYTFTDYEIHWVKQTPVHGLEWIGAIDPETGDTAYTQKFKGKAILTADKSSNTVYMELRSLTSEDSAVYYCTRFYSYAYWGQGTLVTVSA

SEQ ID NO: 10 - protein, 112 aa, synthetic construct
DVVMTQTPLSLPVSLGDQASISCRSSQSLVHTNGHTYLQWYLQKSGQSPKLLIYKVSNRFSGVPDRFSGSGSGTDFTLKISRVEAEDLGVYFCSQSTHVPYTFGGGTKLEIK

SEQ ID NO: 11 - protein, 115 aa, synthetic construct
QVQLQQSGAELVRPGASVTLSCKASGYTFTDYEIHWVKQTPVHGLEWIGAIDPETDNTAYSQKFKGKAILTADKSSSTAYMELRSLTSEDSAVYYCTRYYSYAYWGQGTLVTVSA

SEQ ID NO: 12 - protein, 112 aa, synthetic construct
DVVMTQTPLSLPVSLGDQASISCRSSQSPVHRNGNTYLHWYLQKPGQSPKLLIFKVSNRFSGVPDRFSGSGSGTDFTLKISRVAAEDLGVYFCSQTTHVPYTFGGGTKLEIK

SEQ ID NO: 13 - protein, 5 aa, synthetic construct
DYEMH

SEQ ID NO: 14 - protein, 17 aa, synthetic construct
AIDPETGGTAYNQKFKG

SEQ ID NO: 15 - protein, 6 aa, synthetic construct
YYSYAY

SEQ ID NO: 16 - protein, 16 aa, synthetic construct
RSRQSLVHSNGNTYLQ

SEQ ID NO: 17 - protein, 7 aa, synthetic construct
KVSNRFS

SEQ ID NO: 18 - protein, 9 aa, synthetic construct
FQSIHVPYT

SEQ ID NO: 19 - protein, 17 aa, synthetic construct
AIHPGSGGTAYNQKFKG

SEQ ID NO: 20 - protein, 6 aa, synthetic construct
FYSYAY

SEQ ID NO: 21 - protein, 16 aa, synthetic construct
RSSQSLVHSNGNTYLQ

SEQ ID NO: 22 - protein, 9 aa, synthetic construct
SQSIHVPYT

SEQ ID NO: 23 - protein, 17 aa, synthetic construct
AIGPETGSTAYNQRFKG

SEQ ID NO: 24 - protein, 6 aa, synthetic construct
YYSFAY

SEQ ID NO: 25 - protein, 5 aa, synthetic construct
DYEIH

SEQ ID NO: 26 - protein, 17 aa, synthetic construct
AIDPATGDTAYTQKFKG

SEQ ID NO: 27 - protein, 16 aa, synthetic construct
RSSQSLVHTNGHTYLQ

SEQ ID NO: 28 - protein, 9 aa, synthetic construct
SQSTHVPYT

SEQ ID NO: 29 - protein, 17 aa, synthetic construct
AIDPETGDTAYTQKFKG

SEQ ID NO: 30 - protein, 17 aa, synthetic construct
AIDPETDNTAYSQKFKG

SEQ ID NO: 31 - protein, 16 aa, synthetic construct
RSSQSPVHRNGNTYLH

SEQ ID NO: 32 - protein, 9 aa, synthetic construct
SQTTHVPYT

SEQ ID NO: 33 - protein, 6 aa, synthetic construct
FYSFAY

SEQ ID NO: 34 - protein, 9 aa, synthetic construct
FQSTHVPYT

SEQ ID NO: 35 - protein, 115 aa, synthetic construct
QVQLQQSGAELVRPGASVKLSCKALGYTFTDYEMHWVKQTPVHGLEWIGAIHPGSGGTAYNQKFKGKATLTADKFSSTGYMELSSLTSEDSAVYYCTRYYSYAYWGQGTLVTVSA

SEQ ID NO: 36 - protein, 115 aa, synthetic construct
QVQLVQSGAEVKKPGASVKVSCKASGYTFTDYEMHWVRQAPGQGLEWMGAIHPGSGGTAYNQKFKGRVTMTRDTSTSTVYMELSSLRSEDTAVYYCARYYSYAYWGQGTLVTVSS

SEQ ID NO: 37 - protein, 115 aa, synthetic construct
QVQLVQSGAEVKKPGASVKVSCKASGYTFTDYEMHWVRQAPGQGLEWIGAIHPGSGGTAYNQKFKGRVTMTADTSTSTVYMELSSLRSEDTAVYYCTRYYSYAYWGQGTLVTVSS

SEQ ID NO: 38 - protein, 115 aa, synthetic construct
QVQLVQSGAEVKKPGASVKVSCKALGYTFTDYEMHWVKQAPGQGLEWIGAIHPGSGGTAYNQKFKGRVTLTADTSTSTVYMELSSLRSEDTAVYYCTRYYSYAYWGQGTLVTVSS

SEQ ID NO: 39 - protein, 115 aa, synthetic construct
QVQLVQSGAEVKKPGASVKVSCKALGYTFTDYEMHWVKQAPGQGLEWIGAIHPGSGGTAYNQKFKGRATMTADKFTSTVYMELSSLRSEDTAVYYCTRYYSYAYWGQGTLVTVSS

SEQ ID NO: 40 - protein, 112 aa, synthetic construct
DVVMTQTPLSLPVSLGDQASISCRSSQSLVHSNGNTYLQWYLQKPGQSPKLLIYKVSNRFSGVPDRFSGSGSGTDFILKISRVEAEDLGVYFCFQSIHVPYTFGGGTKLEIK

SEQ ID NO: 41 - protein, 112 aa, synthetic construct
DIVMTQTPLSLSVTPGQPASISCRSSQSLVHSNGNTYLQWYLQKPGQSPQLLIYKVSNRFSGVPDRFSGSGSGTDFTLKISRVEAEDVGVYYCFQSIHVPYTFGGGTKLEIK

SEQ ID NO: 42 - protein, 112 aa, synthetic construct
DIVMTQTPLSLSVTPGQPASISCRSSQSLVHSNGNTYLQWYLQKPGQSPQLLIYKVSNRFSGVPDRFSGSGSGTDFTLKISRVEAEDVGVYFCFQSIHVPYTFGGGTKLEIK

SEQ ID NO: 43 - protein, 112 aa, synthetic construct
DIVMTQTPLSLSVTPGQPASISCRSSQSLVHSNGNTYLQWYLQKPGQSPKLLIYKVSNRFSGVPDRFSGSGSGTDFTLKISRVEAEDVGVYYCFQSIHVPYTFGGGTKLEIK

SEQ ID NO: 44 - protein, 112 aa, synthetic construct
DIVMTQTPLSLSVTPGQPASISCRSSQSLVHSNGNTYLQWYLQKPGQSPKLLIYKVSNRFSGVPDRFSGSGSGTDFTLKISRVEAEDVGVYFCFQSIHVPYTFGGGTKLEIK

SEQ ID NO: 45 - protein, 115 aa, synthetic construct
EVQLVQSGAEVKKPGASVKVSCKASGYTFTDYEMHWVRQAPGQGLEWMGAIHPGSGGTAYNQKFKGRVTMTRDTSISTAYMELSRLRSDDTAVYYCARFYSYAYWGQGTLVTVSS

SEQ ID NO: 46 - protein, 115 aa, synthetic construct
EVQLVQSGAEVKKPGASVKVSCKASGYTFTDYEMHWVRQAPGQGLEWMGAIHPGSGGTAYNQKFKGRVTMTRDTSISTAYMELSRLRSDDTAVYYCTRFYSYAYWGQGTLVTVSS

SEQ ID NO: 47 - protein, 115 aa, synthetic construct
EVQLVQSGAEVKKPGASVKVSCKASGYTFTDYEMHWVRQAPGQGLEWMGAIHPGSGGTAYNQKFKGRVTMTADTSISTAYMELSRLRSDDTAVYYCTRFYSYAYWGQGTLVTVSS

SEQ ID NO: 48 - protein, 115 aa, synthetic construct
EVQLVQSGAEVKKPGASVKVSCKASGYTFTDYEMHWVRQAPGQGLEWMGAIHPGSGGTAYNQKFKGRVTMTADKSISTAYMELSRLRSDDTAVYYCTRFYSYAYWGQGTLVTVSS

SEQ ID NO: 49 - protein, 115 aa, synthetic construct
EVQLVQSGAEVKKPGASVKVSCKASGYTFTDYEMHWVRQAPGQGLEWIGAIHPGSGGTAYNQKFKGRVTLTADKSISTAYMELSRLRSDDTAVYYCTRFYSYAYWGQGTLVTVSS

SEQ ID NO: 50 - protein, 115 aa, synthetic construct
EVQLVQSGAEVKKPGASVKVSCKASGYTFTDYEMHWVRQAPGQGLEWIGAIHPGSGGTAYNQKFKGKATLTADKSISTAYMELSRLRSDDTAVYYCTRFYSYAYWGQGTLVTVSS

SEQ ID NO: 51 - protein, 112 aa, synthetic construct
DVVMTQTPLSLSVTPGQPASISCRSSQSLVHSNGNTYLQWYLQKPGQSPQLLIYKVSNRFSGVPDRFSGSGSGTDFTLKISRVEAEDVGVYYCSQSIHVPYTFGGGTKVEIK

SEQ ID NO: 52 - protein, 112 aa, synthetic construct
DVVMTQTPLSLSVTPGQPASISCRSSQSLVHSNGNTYLQWYLQKPGQSPQLLIYKVSNRFSGVPDRFSGSGSGTDFTLKISRVEAEDVGVYFCSQSIHVPYTFGGGTKVEIK

SEQ ID NO: 53 - protein, 115 aa, synthetic construct
QVQLVQSGAEVKKPGASVKVSCKASGYTFTRYEMHWVRQAPGQGLEWIGAIHPGSGGTAYNSKFKGRVTMTADTSTSTVYMELSSLRSEDTAVYYCTRYYSYAYWGQGTLVTVSS

SEQ ID NO: 54 - protein, 112 aa, synthetic construct
DIVMTQTPLSLSVTPGQPASISCRSSQSLVHSNGNTYLQWYLQKPGQSPKLLIYKVSNRYSGVPDRFSGSGSGTDFTLKISRVEAEDVGVYYCVESIHVPYTFGGGTKLEIK

SEQ ID NO: 55 - protein, 115 aa, synthetic construct
QVQLVQSGAEVKKPGASVKVSCKASGYTFTGYEMHWVRQAPGQGLEWIGAIHPGSGGTAYNQKFKGRVTMTADTSTSTVYMELSSLRSEDTAVYYCTRYYSYAYWGQGTLVTVSS

SEQ ID NO: 56 - protein, 112 aa, synthetic construct
DIVMTQTPLSLSVTPGQPASISCRSSQSLVHSNGNTYLQWYLQKPGQSPKLLIYKVSNRFAGVPDRFSGSGSGTDFTLKISRVEAEDVGVYYCVESIHVPYTFGGGTKLEIK

SEQ ID NO: 57 - protein, 115 aa, synthetic construct
QVQLVQSGAEVKKPGASVKVSCKASGYRFTDYEMHWVRQAPGQGLEWIGAIHPGSGGTAYNQLFKGRVTMTADTSTSTVYMELSSLRSEDTAVYYCTRYYSYAYWGQGTLVTVSS

SEQ ID NO: 58 - protein, 112 aa, synthetic construct
DIVMTQTPLSLSVTPGQPASISCRSSQSLVHSNGNTYLQWYLQKPGQSPKLLIYKVSNRFPGVPDRFSGSGSGTDFTLKISRVEAEDVGVYYCVESIHVPYTFGGGTKLEIK

SEQ ID NO: 59 - protein, 5 aa, synthetic construct
RYEMH

SEQ ID NO: 60 - protein, 17 aa, synthetic construct
AIHPGSGGTAYNSKFKG

SEQ ID NO: 61 - protein, 7 aa, synthetic construct
KVSNRYS

SEQ ID NO: 62 - protein, 9 aa, synthetic construct
VESIHVPYT

SEQ ID NO: 63 - protein, 5 aa, synthetic construct
GYEMH

SEQ ID NO: 64 - protein, 7 aa, synthetic construct
KVSNRFA

SEQ ID NO: 65 - protein, 17 aa, synthetic construct
AIHPGSGGTAYNQLFKG

SEQ ID NO: 66 - protein, 7 aa, synthetic construct
KVSNRFP

SEQ ID NO: 67 - protein, 115 aa, synthetic construct
QVQLQQSGAELVRPGASVKLSCKALGYTFTDYEMHWVKQTPVHGLEWIGAIHPGSGGTAYNQKFKGKATLTADKFSSTGYMELSSLTSEDSAVYYCTRFYSFAYWGQGTLVTVSA

SEQ ID NO: 68 - protein, 112 aa, synthetic construct
DVVMTQTPLSLPVSLGDQASISCRSSQSLVHSNGNTYLQWYLQKPGQSPKLLIYKVSNRFSGVPDRFSGSGSGTDFILKISRVEAEDLGVYFCSQSTHVPYTFGGGTKLEIK

SEQ ID NO: 69 - protein, 115 aa, synthetic construct
QVQLQQSGAELVRPGASVKLSCKALGYTFTDYEMHWVKQTPVHGLEWIGAIHPGSGGTAYNQKFKGKATLTADKFSSTGYMELSSLTSEDSAVYYCTRYYSFAYWGQGTLVTVSA

SEQ ID NO: 70 - protein, 112 aa, synthetic construct
DVVMTQTPLSLPVSLGDQASISCRSSQSLVHSNGNTYLQWYLQKPGQSPKLLIYKVSNRFSGVPDRFSGSGSGTDFILKISRVEAEDLGVYFCFQSTHVPYTFGGGTKLEIK

SEQ ID NO: 71 - skipped

SEQ ID NO: 72 - protein, 17 aa, synthetic construct
  VARIANT 3: note = X is D, G, or H
  VARIANT 5: note = X is A, E or G
  VARIANT 6: note = X is S or T
  VARIANT 7: note = X is D or G
  VARIANT 8: note = X is D, G, N or S
  VARIANT 12: note = N, S or T
  VARIANT 13: note = X is Q or S
  VARIANT 14: note = X is R, K or L
AIXPXXXXTAYXXXFKG

SEQ ID NO: 73 - protein, 6 aa, synthetic construct
  VARIANT 1: note = F or Y
  VARIANT 4: note = X is F or Y
XYSXAY

SEQ ID NO: 74 - protein, 16 aa, synthetic construct
  VARIANT 3: note = X is R or S
  VARIANT 6: note = X is L or P
  VARIANT 9: note = X is S, R or T
  VARIANT 12: note = X is H or N
  VARIANT 16: note = X is H or Q
RSXQSXVHXNGXTYLX

SEQ ID NO: 75 - protein, 7 aa, synthetic construct
  VARIANT 6: note = X is F or Y
  VARIANT 7: note = X is S, A or P
KVSNRXX

SEQ ID NO: 76 - protein, 9 aa, synthetic construct
  VARIANT 1: note = X is F, S or V
  VARIANT 2: note = X is Q or E
  VARIANT 3: note = X is S or T
  VARIANT 4: note = X is I or T
XXXXHVPYT